European Patent Application EP 4 537 856 A1, published April 16, 2025. Title: Adeno-Associated Virus Pharmaceutical Composition and Use Thereof. Applicant: Chengdu Origen Biotechnology Co., Ltd. The sequence listing filed with the application follows.

SEQUENCE LISTING (9 sequences)

SEQ ID NO: 1 - protein, 431 aa, synthetic construct
SDTGRPFVEMYSEIPEIIHMTEGRELVIPCRVTSPNITVTLKKFPLDTLIPDGKRIIWDSRKGFIISNATYKEIGLLTCEATVNGHLYKTNYLTHRQTNTIIDVVLSPSHGIELSVGEKLVLNCTARTELNVGIDFNWEYPSSKHQHKKLVNRDLKTQSGSEMKKFLSTLTIDGVTRSDQGLYTCAASSGLMTKKNSTFVRVHEKDKTHTCPPCPAPELLGGPSVFLFPPKPKDTLMISRTPEVTCVVVDVSHEDPEVKFNWYVDGVEVHNAKTKPREEQYNSTYRVVSVLTVLHQDWLNGKEYKCKVSNKALPAPIEKTISKAKGQPREPQVYTLPPSRDELTKNQVSLTCLVKGFYPSDIAVEWESNGQPENNYKTTPPVLDSDGSFFLYSKLTVDKSRWQQGNVFSCSVMHEALHNHYTQKSLSLSPG

SEQ ID NO: 2 - protein, 526 aa, synthetic construct
GRPFVEMYSEIPEIIHMTEGRELVIPCRVTSPNITVTLKKFPLDTLIPDGKRIIWDSRKGFIISNATYKEIGLLTCEATVNGHLYKTNYLTHRQTNTIIDVVLSPSHGIELSVGEKLVLNCTARTELNVGIDFNWEYPSSKHQHKKLVNRDLKTQSGSEMKKFLSTLTIDGVTRSDQGLYTCAASSGLMTKKNSTFVRVHEKPFVAFGSGMESLVEATVGERVRIPAKYLGYPPPEIKWYKNGIPLESNHTIKAGHVLTIMEVSERDTGNYTVILTNPISKEKQSHVVSLVVYVPPGPGDKTHTCPLCPAPELLGGPSVFLFPPKPKDTLMISRTPEVTCVVVDVSHEDPEVKFNWYVDGVEVHNAKTKPREEQYNSTYRVVSVLTVLHQDWLNGKEYKCKVSNKALPAPIEKTISKAKGQPREPQVYTLPPSRDELTKNQVSLTCLVKGFYPSDIAVEWESNGQPENNYKATPPVLDSDGSFFLYSKLTVDKSRWQQGNVFSCSVMHEALHNHYTQKSLSLSPGK

SEQ ID NO: 3 - protein, 123 aa, synthetic construct [sequence omitted]

SEQ ID NO: 4 - protein, 124 aa, synthetic construct
DIQLTQSPSSLSASVGDRVTITCSASQDISNYLNWYQQKPGKAPKVLIYFTSSLHSGVPSRFSGSGSGTDFTLTISSLQPEDFATYYCQQYSTVPWTFGQGTKVEIKRTVAAPSVFIFPPSDEQ

SEQ ID NO: 5 - protein, 120 aa, synthetic construct
EVQLVESGGGLVQPGGSLRLSCTASGFSLTDYYYMTWVRQAPGKGLEWVGFIDPDDDPYYATWAKGRFTISRDNSKNTLYLQMNSLRAEDTAVYYCAGGDHNSGWGLDIWGQGTLVTVSS

SEQ ID NO: 6 - protein, 112 aa, synthetic construct
MEIVMTQSPSTLSASVGDRVIITCQASEIIHSWLAWYQQKPGKAPKLLIYLASTLASGVPSRFSGSGSGAEFTLTISSLQPDDFATYYCQNVYLASTNGANFGQGTKLTVLG

SEQ ID NO: 7 - protein, 252 aa, synthetic construct
MEIVMTQSPSTLSASVGDRVIITCQASEIIHSWLAWYQQKPGKAPKLLIYLASTLASGVPSRFSGSGSGAEFTLTISSLQPDDFATYYCQNVYLASTNGANFGQGTKLTVLGGGGGSGGGGSGGGGSGGGGSEVQLVESGGGLVQPGGSLRLSCTASGFSLTDYYYMTWVRQAPGKGLEWVGFIDPDDDPYYATWAKGRFTISRDNSKNTLYLQMNSLRAEDTAVYYCAGGDHNSGWGLDIWGQGTLVTVSS

SEQ ID NO: 8 - DNA, 1659 bp, synthetic construct
  source 1..1659: mol_type = other DNA
atggtcagctactgggacaccggggtcctgctgtgcgcgctgctcagctgtctgcttctcacaggatctagttccggaggtagacctttcgtagagatgtacagtgaaatccccgaaattatacacatgactgaaggaagggagctcgtcattccctgccgggttacgtcacctaacatcactgttactttaaaaaagtttccacttgacactttgatccctgatggaaaacgcataatctgggacagtagaaagggcttcatcatatcaaatgcaacgtacaaagaaatagggcttctgacctgtgaagcaacagtcaatgggcatttgtataagacaaactatctcacacatcgacaaaccaatacaatcatagatgtggttctgagtccgtctcatggaattgaactatctgttggagaaaagcttgtcttaaattgtacagcaagaactgaactaaatgtggggattgacttcaactgggaatacccttcttcgaagcatcagcataagaaacttgtaaaccgagacctaaaaacccagtctgggagtgagatgaagaaatttttgagcaccttaactatagatggtgtaacccggagtgaccaaggattgtacacctgtgcagcatccagtgggctgatgaccaagaagaacagcacatttgtcagggtccatgaaaaaccttttgttgcttttggaagtggcatggaatctctggtggaagccacggtgggggagcgtgtcagaatccctgcgaagtaccttggttacccacccccagaaataaaatggtataaaaatggaataccccttgagtccaatcacacaattaaagcggggcatgtactgacgattatggaagtgagtgaaagagacacaggaaattacactgtcatccttaccaatcccatttcaaaggagaagcagagccatgtggtctctctggttgtgtatgtcccaccgggcccgggcgacaaaactcacacatgcccactgtgcccagcacctgaactcctggggggaccgtcagtcttcctcttccccccaaaacccaaggacaccctcatgatctcccggacccctgaggtcacatgcgtggtggtggacgtgagccacgaagaccctgaggtcaagttcaactggtacgtggacggcgtggaggtgcataatgccaagacaaagccgcgggaggagcagtacaacagcacgtaccgtgtggtcagcgtcctcaccgtcctgcaccaggactggctgaatggcaaggagtacaagtgcaaggtctccaacaaagccctcccagcccccatcgagaaaaccatctccaaagccaaagggcagccccgagaaccacaggtgtacaccctgcccccatcccgggatgagctgaccaagaaccaggtcagcctgacctgcctagtcaaaggcttctatcccagcgacatcgccgtggagtgggagagcaatgggcagccggagaacaactacaaggccacgcctcccgtgctggactccgacggctccttcttcctctacagcaagctcaccgtggacaagagcaggtggcagcaggggaacgtcttctcatgctccgtgatgcatgaggctctgcacaaccactacacgcagaagagcctctccctgtctccgggtaaatga

SEQ ID NO: 9 - DNA, 4009 bp, synthetic construct
  source 1..4009: mol_type = other DNA
ctgcgcgctcgctcgctcactgaggccgcccgggcaaagcccgggcgtcgggcgacctttggtcgcccggcctcagtgagcgagcgagcgcgcagagagggagtggccaactccatcactaggggttccttgtagttaatgattaacccgccatgctacttatctaccagggtaatggggatcctctagaactatagctagtcgacattgattattgactagttattaatagtaatcaattacggggtcattagttcatagcccatatatggagttccgcgttacataacttacggtaaatggcccgcctggctgaccgcccaacgacccccgcccattgacgtcaataatgacgtatgttcccatagtaacgccaatagggactttccattgacgtcaatgggtggagtatttacggtaaactgcccacttggcagtacatcaagtgtatcatatgccaagtacgccccctattgacgtcaatgacggtaaatggcccgcctggcattatgcccagtacatgaccttatgggactttcctacttggcagtacatctacgtattagtcatcgctattaccatggtcgaggtgagccccacgttctgcttcactctccccatctcccccccctccccacccccaattttgtatttatttattttttaattattttgtgcagcgatgggggcggggggggggggggggcgcgcgccaggcggggcggggcggggcgaggggcggggcggggcgaggcggagaggtgcggcggcagccaatcagagcggcgcgctccgaaagtttccttttatggcgaggcggcggcggcggcggccctataaaaagcgaagcgcgcggcgggcgggagtcgctgcgcgctgccttcgccccgtgccccgctccgccgccgcctcgcgccgcccgccccggctctgactgaccgcgttactcccacaggtgagcgggcgggacggcccttctcctccgggctgtaattagcgcttggtttaatgacggcttgtttcttttctgtggctgcgtgaaagccttgaggggctccgggagggccctttgtgcggggggagcggctcggggggtgcgtgcgtgtgtgtgtgcgtggggagcgccgcgtgcggctccgcgctgcccggcggctgtgagcgctgcgggcgcggcgcggggctttgtgcgctccgcagtgtgcgcgaggggagcgcggccgggggcggtgccccgcggtgcggggggggctgcgaggggaacaaaggctgcgtgcggggtgtgtgcgtgggggggtgagcagggggtgtgggcgcgtcggtcgggctgcaaccccccctgcacccccctccccgagttgctgagcacggcccggcttcgggtgcggggctccgtacggggcgtggcgcggggctcgccgtgccgggcggggggtggcggcaggtgggggtgccgggcggggcggggccgcctcgggccggggagggctcgggggaggggcgcggcggcccccggagcgccggcggctgtcgaggcgcggcgagccgcagccattgccttttatggtaatcgtgcgagagggcgcagggacttcctttgtcccaaatctgtgcggagccgaaatctgggaggcgccgccgcaccccctctagcgggcgcggggcgaagcggtgcggcgccggcaggaaggaaatgggcggggagggccttcgtgcgtcgccgcgccgccgtccccttctccctctccagcctcggggctgtccgcggggggacggctgccttcgggggggacggggcagggcggggttcggcttctggcgtgtgaccggcggctctagagcctctgctaaccatgttcatgccttcttctttttcctacagctcctgggcaacgtgctggttattgtgctgtctcatcattttggcaaagaattcgccaccatggtcagctactgggacaccggggtcctgctgtgcgcgctgctcagctgtctgcttctcacaggatctagttccggaggtagacctttcgtagagatgtacagtgaaatccccgaaattatacacatgactgaaggaagggagctcgtcattccctgccgggttacgtcacctaacatcactgttactttaaaaaagtttccacttgacactttgatccctgatggaaaacgcataatctgggacagtagaaagggcttcatcatatcaaatgcaacgtacaaagaaatagggcttctgacctgtgaagcaacagtcaatgggcatttgtataagacaaactatctcacacatcgacaaaccaatacaatcatagatgtggttctgagtccgtctcatggaattgaactatctgttggagaaaagcttgtcttaaattgtacagcaagaactgaactaaatgtggggattgacttcaactgggaatacccttcttcgaagcatcagcataagaaacttgtaaaccgagacctaaaaacccagtctgggagtgagatgaagaaatttttgagcaccttaactatagatggtgtaacccggagtgaccaaggattgtacacctgtgcagcatccagtgggctgatgaccaagaagaacagcacatttgtcagggtccatgaaaaaccttttgttgcttttggaagtggcatggaatctctggtggaagccacggtgggggagcgtgtcagaatccctgcgaagtaccttggttacccacccccagaaataaaatggtataaaaatggaataccccttgagtccaatcacacaattaaagcggggcatgtactgacgattatggaagtgagtgaaagagacacaggaaattacactgtcatccttaccaatcccatttcaaaggagaagcagagccatgtggtctctctggttgtgtatgtcccaccgggcccgggcgacaaaactcacacatgcccactgtgcccagcacctgaactcctggggggaccgtcagtcttcctcttccccccaaaacccaaggacaccctcatgatctcccggacccctgaggtcacatgcgtggtggtggacgtgagccacgaagaccctgaggtcaagttcaactggtacgtggacggcgtggaggtgcataatgccaagacaaagccgcgggaggagcagtacaacagcacgtaccgtgtggtcagcgtcctcaccgtcctgcaccaggactggctgaatggcaaggagtacaagtgcaaggtctccaacaaagccctcccagcccccatcgagaaaaccatctccaaagccaaagggcagccccgagaaccacaggtgtacaccctgcccccatcccgggatgagctgaccaagaaccaggtcagcctgacctgcctagtcaaaggcttctatcccagcgacatcgccgtggagtgggagagcaatgggcagccggagaacaactacaaggccacgcctcccgtgctggactccgacggctccttcttcctctacagcaagctcaccgtggacaagagcaggtggcagcaggggaacgtcttctcatgctccgtgatgcatgaggctctgcacaaccactacacgcagaagagcctctccctgtctccgggtaaatgaacgcgtggtacctctagagtcgacccgggcggcctcgaggacggggtgaactacgcctgaggatccgatctttttccctctgccaaaaattatggggacatcatgaagccccttgagcatctgacttctggctaataaaggaaatttattttcattgcaatagtgtgttggaattttttgtgtctctcactcggaagcaattcgttgatctgaatttcgaccacccataatacccattaccctggtagataagtagcatggcgggttaatcattaactacaaggaacccctagtgatggagttggccactccctctctgcgcgctcgctcgctcactgaggccgggcgaccaaaggtcgcccgacgcccgggctttgcccgggcggcctcagtgagcgagcgagcgcgcag